European Patent Application EP 4 548 780 A1, published May 7, 2025. Title: FPR2 agonist comprising outer membrane vesicle derived from lactic acid bacterium. Applicant: Asahi Group Holdings, Ltd. Application JP. The sequence listing filed with the application follows.

SEQUENCE LISTING (3 sequences)

SEQ ID NO: 1 - protein, 6 aa, synthetic construct
  REGION 1..6: note = peptide
WKYMVM

SEQ ID NO: 2 - protein, 6 aa, synthetic construct
  REGION 1..6: note = peptide
  MOD_RES 6: note = D-Met
WKYMVM

SEQ ID NO: 3 - protein, 6 aa, synthetic construct
  REGION 1..6: note = peptide
WRWWWW